European Patent Application EP 4 276 111 A1, published November 15, 2023. Title: ANTIBODY SPECIFICALLY BINDING TO 4-1BB AND ANTIGEN-BINDING FRAGMENT OF ANTIBODY. Applicant: BEIJING HANMI PHARMACEUTICAL CO., LTD. The sequence listing filed with the application follows.

SEQUENCE LISTING (33 sequences)

SEQ ID NO: 1 - protein, 11 aa, Artificial Sequence
  LCDR1
RASQDISNYLN

SEQ ID NO: 2 - protein, 7 aa, Artificial Sequence
  LCDR2
HTSRLHS

SEQ ID NO: 3 - protein, 9 aa, Artificial Sequence
  LCDR3
QQGHTLPRT

SEQ ID NO: 4 - protein, 10 aa, Artificial Sequence
  HCDR1
GYTFTSYWIN

SEQ ID NO: 5 - protein, 17 aa, Artificial Sequence
  HCDR2
NIYPSDSYTNYNQKFKD

SEQ ID NO: 6 - protein, 10 aa, Artificial Sequence
  HCDR3
LYYGSSPFDY

SEQ ID NO: 7 - protein, 107 aa, Artificial Sequence
  Chimeric antibody light chain variable region
DIQMTQTTSSLSASLGDRVTISCRASQDISNYLNWYQQKPDGTVKLLIYHTSRLHSGVPPRFSGSGSGTNYSLTISNLEQEDIATYFCQQGHTLPRTFGGGTKLEIK

SEQ ID NO: 8 - protein, 119 aa, Artificial Sequence
  Chimeric antibody heavy chain variable region
QVQLQQPGAELVRPGASMKLSCKASGYTFTSYWINWVKQRPGQGLEWIGNIYPSDSYTNYNQKFKDKATLTVDKSSSTAYMQLSSPTSEDSAVYYCTRLYYGSSPFDYWGQGTTLTVSS

SEQ ID NO: 9 - protein, 107 aa, Artificial Sequence [sequence omitted]

SEQ ID NO: 10 - protein, 327 aa, Artificial Sequence
  Heavy chain constant region
ASTKGPSVFPLAPCSRSTSESTAALGCLVKDYFPEPVTVSWNSGALTSGVHTFPAVLQSSGLYSLSSVVTVPSSSLGTKTYTCNVDHKPSNTKVDKRVESKYGPPCPPCPAPEFLGGPSVFLFPPKPKDTLMISRTPEVTCVVVDVSQEDPEVQFNWYVDGVEVHNAKTKPREEQFNSTYRVVSVLTVLHQDWLNGKEYKCKVSNKGLPSSIEKTISKAKGQPREPQVYTLPPSQEEMTKNQVSLTCLVKGFYPSDIAVEWESNGQPENNYKTTPPVLDSDGSFFLYSRLTVDKSRWQEGNVFSCSVMHEALHNHYTQKSLSLSLGK

SEQ ID NO: 11 - protein, 107 aa, Artificial Sequence
  Humanized antibody light chain variable region
DIQMTQSPSSLSASVGDRVTITCRASQDISNYLNWYQQKPGKVPKLLIYHTSRLHSGVPSRFSGSGSGTDFTLTISSLQPEDVATYYCQQGHTLPRTFGGGTKVEIK

SEQ ID NO: 12 - protein, 119 aa, Artificial Sequence
  Humanized antibody heavy chain variable region
QVQLVQSGAEVKKPGSSVKVSCKASGYTFTSYWINWVRQAPGQGLEWMGNIYPSDSYTNYNQKFKDRVTITADKSTSTAYMELSSLRSEDTAVYYCARLYYGSSPFDYWGQGTTVTVSS

SEQ ID NO: 13 - protein, 107 aa, Artificial Sequence
  Humanized antibody light chain variable region
DIQMTQSPSSLSASVGDRVTITCRASQDISNYLNWYQQKPGKVPKLLIYHTSRLHSGVPSRFSGSGSGTDYTLTISSLQPEDVATYYCQQGHTLPRTFGGGTKVEIK

SEQ ID NO: 14 - protein, 107 aa, Artificial Sequence
  Humanized antibody light chain variable region
DIQMTQSPSSLSASVGDRVTITCRASQDISNYLNWYQQKPGKTPKLLIYHTSRLHSGVPSRFSGSGSGTDYTLTISSLQPEDVATYYCQQGHTLPRTFGGGTKVEIK

SEQ ID NO: 15 - protein, 107 aa, Artificial Sequence
  Humanized antibody light chain variable region
DIQMTQSPSSLSASVGDRVTITCRASQDISNYLNWYQQKPGKVPKLLIYHTSRLHSGVPSRFSGSGSGTDYTLTISSLQPEDVATYFCQQGHTLPRTFGGGTKVEIK

SEQ ID NO: 16 - protein, 107 aa, Artificial Sequence
  Humanized antibody light chain variable region
DIQMTQSPSSLSASVGDRVTITCRASQDISNYLNWYQQKPGKTPKLLIYHTSRLHSGVPSRFSGSGSGTDYTLTISSLQPEDVATYFCQQGHTLPRTFGGGTKVEIK

SEQ ID NO: 17 - protein, 107 aa, Artificial Sequence
  Humanized antibody light chain variable region
DIQMTQSPSSLSASVGDRVTITCRASQDISNYLNWYQQKPGKTPKLLIYHTSRLHSGVPSRFSGSGSGTDFTLTISSLQPEDVATYFCQQGHTLPRTFGGGTKVEIK

SEQ ID NO: 18 - protein, 107 aa, Artificial Sequence
  Humanized antibody light chain variable region
DIQMTQSPSSLSASVGDRVTITCRASQDISNYLNWYQQKPGKTVKLLIYHTSRLHSGVPSRFSGSGSGTDYTLTISSLQPEDVATYYCQQGHTLPRTFGGGTKVEIK

SEQ ID NO: 19 - protein, 107 aa, Artificial Sequence
  Humanized antibody light chain variable region
DIQMTQSPSSLSASVGDRVTITCRASQDISNYLNWYQQKPGKTPKLLIYHTSRLHSGVPPRFSGSGSGTDYTLTISSLQPEDVATYYCQQGHTLPRTFGGGTKVEIK

SEQ ID NO: 20 - protein, 107 aa, Artificial Sequence
  Humanized antibody light chain variable region
DIQMTQSPSSLSASVGDRVTITCRASQDISNYLNWYQQKPGKTVKLLIYHTSRLHSGVPPRFSGSGSGTDYTLTISSLQPEDVATYYCQQGHTLPRTFGGGTKVEIK

SEQ ID NO: 21 - protein, 119 aa, Artificial Sequence
  Humanized antibody heavy chain variable region
QVQLVQSGAEVKKPGSSVKVSCKASGYTFTSYWINWVRQAPGQGLEWMGNIYPSDSYTNYNQKFKDRVTITADKSTSTAYMELSSLRSEDTAVYYCTRLYYGSSPFDYWGQGTTVTVSS

SEQ ID NO: 22 - protein, 119 aa, Artificial Sequence
  Humanized antibody heavy chain variable region
QVQLVQSGAEVKKPGSSVKVSCKASGYTFTSYWINWVRQAPGQGLEWMGNIYPSDSYTNYNQKFKDRVTITVDKSTSTAYMELSSLRSEDTAVYYCTRLYYGSSPFDYWGQGTTVTVSS

SEQ ID NO: 23 - protein, 119 aa, Artificial Sequence
  Humanized antibody heavy chain variable region
QVQLVQSGAEVKKPGSSVKLSCKASGYTFTSYWINWVRQAPGQGLEWMGNIYPSDSYTNYNQKFKDRVTITVDKSTSTAYMELSSLRSEDTAVYYCTRLYYGSSPFDYWGQGTTVTVSS

SEQ ID NO: 24 - protein, 119 aa, Artificial Sequence
  Humanized antibody heavy chain variable region
QVQLVQSGAEVKKPGSSVKVSCKASGYTFTSYWINWVRQAPGQGLEWIGNIYPSDSYTNYNQKFKDRVTITVDKSTSTAYMELSSLRSEDTAVYYCTRLYYGSSPFDYWGQGTTVTVSS

SEQ ID NO: 25 - protein, 119 aa, Artificial Sequence
  Humanized antibody heavy chain variable region
QVQLVQSGAEVKKPGSSVKVSCKASGYTFTSYWINWVRQAPGQGLEWMGNIYPSDSYTNYNQKFKDRVTLTVDKSTSTAYMELSSLRSEDTAVYYCTRLYYGSSPFDYWGQGTTVTVSS

SEQ ID NO: 26 - protein, 119 aa, Artificial Sequence
  Humanized antibody heavy chain variable region
QVQLVQSGAEVKKPGSSVKLSCKASGYTFTSYWINWVRQAPGQGLEWIGNIYPSDSYTNYNQKFKDRVTLTVDKSTSTAYMELSSLRSEDTAVYYCTRLYYGSSPFDYWGQGTTVTVSS

SEQ ID NO: 27 - protein, 119 aa, Artificial Sequence
  Humanized antibody heavy chain variable region
QVQLVQSGAEVKKPGSSVKVSCKASGYTFTSYWINWVRQAPGQGLEWIGNIYPSDSYTNYNQKFKDRVTLTVDKSTSTAYMELSSLRSEDTAVYYCTRLYYGSSPFDYWGQGTTVTVSS

SEQ ID NO: 28 - protein, 119 aa, Artificial Sequence
  Humanized antibody heavy chain variable region
QVQLVQSGAEVKKPGSSVKLSCKASGYTFTSYWINWVRQAPGQGLEWMGNIYPSDSYTNYNQKFKDRVTLTVDKSTSTAYMELSSLRSEDTAVYYCTRLYYGSSPFDYWGQGTTVTVSS

SEQ ID NO: 29 - protein, 119 aa, Artificial Sequence
  Humanized antibody heavy chain variable region
QVQLVQSGAEVKKPGSSVKLSCKASGYTFTSYWINWVRQAPGQGLEWIGNIYPSDSYTNYNQKFKDRVTITVDKSTSTAYMELSSLRSEDTAVYYCTRLYYGSSPFDYWGQGTTVTVSS

SEQ ID NO: 30 - protein, 119 aa, Artificial Sequence
  Humanized antibody heavy chain variable region
QVQLVQSGAEVKKPGSSVKLSCKASGYTFTSYWINWVRQAPGQGLEWIGNIYPSDSYTNYNQKFKDRVTLTADKSTSTAYMELSSLRSEDTAVYYCTRLYYGSSPFDYWGQGTTVTVSS

SEQ ID NO: 31 - protein, 119 aa, Artificial Sequence
  Humanized antibody heavy chain variable region
QVQLVQSGAEVKKPGSSVKLSCKASGYTFTSYWINWVRQAPGQGLEWIGNIYPSDSYTNYNQKFKDRVTLTVDKSTSTAYMELSSLRSEDTAVYYCARLYYGSSPFDYWGQGTTVTVSS

SEQ ID NO: 32 - DNA, 47 bp, Artificial Sequence
  VHGSP
gattacgccaagcttgccagtggatagacaagcttgggtgtcgtttt

SEQ ID NO: 33 - DNA, 42 bp, Artificial Sequence
  VLGSP
gattacgccaagcttgatggatccagttggtgcagcatcagc